European Patent Application EP 4 257 614 A2, published October 11, 2023. Title: Pharmaceutical Combinations. Applicant: Berlin-Chemie AG. Application EP. The sequence listing filed with the application follows.

SEQUENCE LISTING (207 sequences)

SEQ ID NO: 1 - protein, 119 aa, Homo sapiens
EVQLVESGGGLVKPGGSLRLSCAASGFTYSNAWMSWVRQAPGKGLEWVGRIKSKTDGGTTDYAAPVQGRFTISRDDSKNTLYLQMNSLKTEDTAVYYCTIFGVVSFDYWGQGTLVTVSS

SEQ ID NO: 2 - protein, 108 aa, Homo sapiens
DVQMTQSPSSLSASVGDRVTITCRASQSISDYLSWYQQRPGKAPNLLIYAASNLKTGVPSRFSGSGSGTDFTLTISTLQPEDFATYYCQQSYRSPWTFGQGTKVEIKR

SEQ ID NO: 3 - DNA, 357 bp, Homo sapiens
  source 1..357: mol_type = other DNA
gaggtgcagctggtggagtctgggggaggcttggtaaagccgggggggtcccttagactctcctgtgcagcctctggcttcacttacagtaacgcctggatgagctgggtccgccaggctccagggaaggggctggagtgggttggccgtattaaaagcaaaactgatggtgggacaacagactacgctgcacccgtgcaaggcagattcaccatctcaagagatgattcaaaaaacacgctgtatctgcaaatgaacagcctgaaaaccgaggacacagccgtgtattactgtacgatttttggagtggttagctttgactactggggccagggaaccctggtcaccgtctcctca

SEQ ID NO: 4 - DNA, 324 bp, Homo sapiens
  source 1..324: mol_type = other DNA
gacgtccagatgacccagtctccatcctccctgtctgcatctgttggagacagagtcaccatcacttgccgggcaagtcagagcattagcgactatttaagttggtatcagcagagaccagggaaagcccctaacctcctgatctatgctgcatccaatttaaagactggggtcccatcaaggttcagtggcagtggatctgggacagatttcactctcaccatcagcactctgcaacctgaagattttgcaacgtactactgtcaacagagttacaggtccccgtggacgttcggccaagggaccaaggtggaaatcaaacga

SEQ ID NO: 5 - protein, 5 aa, Homo sapiens
NAWMS

SEQ ID NO: 6 - protein, 19 aa, Homo sapiens
RIKSKTDGGTTDYAAPVQG

SEQ ID NO: 7 - protein, 8 aa, Homo sapiens
FGVVSFDY

SEQ ID NO: 8 - protein, 11 aa, Homo sapiens
RASQSISDYLS

SEQ ID NO: 9 - protein, 7 aa, Homo sapiens
AASNLKT

SEQ ID NO: 10 - protein, 9 aa, Homo sapiens
QQSYRSPWT

SEQ ID NO: 11 - protein, 104 aa, Homo sapiens
EVQLVESGGGLVKPGGSLRLSCAASGFTFSNAWMSWVRQAPGKGLEWVGRIKSKTDGGTTDYAAPVKGRFTISRDDSKNTLYLQMNSLKTEDTAVYYCTTTTVT

SEQ ID NO: 12 - protein, 15 aa, Homo sapiens
YFDYWGQGTLVTVSS

SEQ ID NO: 13 - protein, 93 aa, Homo sapiens
DIQMTQSPSSLSASVGDRVTITCRASQSISSYLNWYQQKPGKAPKLLIYAASSLQSGVPSRFSGSGSGTDFTLTISSLQPEDFATYYCQQSYS

SEQ ID NO: 14 - protein, 13 aa, Homo sapiens
WTFGQGTKVEIKR

SEQ ID NO: 15 - protein, 1722 aa, Homo sapiens
MRTGWATPRRPAGLLMLLFWFFDLAEPSGRAANDPFTIVHGNTGKCIKPVYGWIVADDCDETEDKLWKWVSQHRLFHLHSQKCLGLDITKSVNELRMFSCDSSAMLWWKCEHHSLYGAARYRLALKDGHGTAISNASDVWKKGGSEESLCDQPYHEIYTRDGNSYGRPCEFPFLIDGTWHHDCILDEDHSGPWCATTLNYEYDRKWGICLKPENGCEDNWEKNEQFGSCYQFNTQTALSWKEAYVSCQNQGADLLSINSAAELTYLKEKEGIAKIFWIGLNQLYSARGWEWSDHKPLNFLNWDPDRPSAPTIGGSSCARMDAESGLWQSFSCEAQLPYVCRKPLNNTVELTDVWTYSDTRCDAGWLPNNGFCYLLVNESNSWDKAHAKCKAFSSDLISIHSLADVEVVVTKLHNEDIKEEVWIGLKNINIPTLFQWSDGTEVTLTYWDENEPNVPYNKTPNCVSYLGELGQWKVQSCEEKLKYVCKRKGEKLNDASSDKMCPPDEGWKRHGETCYKIYEDEVPFGTNCNLTITSRFEQEYLNDLMKKYDKSLRKYFWTGLRDVDSCGEYNWATVGGRRRAVTFSNWNFLEPASPGGCVAMSTGKSVGKWEVKDCRSFKALSICKKMSGPLGPEEASPKPDDPCPEGWQSFPASLSCYKVFHAERIVRKRNWEEAERFCQALGAHLSSFSHVDEIKEFLHFLTDQFSGQHWLWIGLNKRSPDLQGSWQWSDRTPVSTIIMPNEFQQDYDIRDCAAVKVFHRPWRRGWHFYDDREFIYLRPFACDTKLEWVCQIPKGRTPKTPDWYNPDRAGIHGPPLIIEGSEYWFVADLHLNYEEAVLYCASNHSFLATITSFVGLKAIKNKIANISGDGQKWWIRISEWPIDDHFTYSRYPWHRFPVTFGEECLYMSAKTWLIDLGKPTDCSTKLPFICEKYNVSSLEKYSPDSAAKVQCSEQWIPFQNKCFLKIKPVSLTFSQASDTCHSYGGTLPSVLSQIEQDFITSLLPDMEATLWIGLRWTAYEKINKWTDNRELTYSNFHPLLVSGRLRIPENFFEEESRYHCALILNLQKSPFTGTWNFTSCSERHFVSLCQKYSEVKSRQTLQNASETVKYLNNLYKIIPKTLTWHSAKRECLKSNMQLVSITDPYQQAFLSVQALLHNSSLWIGLFSQDDELNFGWSDGKRLHFSRWAETNGQLEDCVVLDTDGFWKTVDCNDNQPGAICYYSGNETEKEVKPVDSVKCPSPVLNTPWIPFQNCCYNFIITKNRHMATTQDEVHTKCQKLNPKSHILSIRDEKENNFVLEQLLYFNYMASWVMLGITYRNKSLMWFDKTPLSYTHWRAGRPTIKNEKFLAGLSTDGFWDIQTFKVIEEAVYFHQHSILACKIEMVDYKEEYNTTLPQFMPYEDGIYSVIQKKVTWYEALNMCSQSGGHLASVHNQNGQLFLEDIVKRDGFPLWVGLSSHDGSESSFEWSDGSTFDYIPWKGQTSPGNCVLLDPKGTWKHEKCNSVKDGAICYKPTKSKKLSRLTYSSRCPAAKENGSRWIQYKGHCYKSDQALHSFSEAKKLCSKHDHSATIVSIKDEDENKFVSRLMRENNNITMRVWLGLSQHSVDQSWSWLDGSEVTFVKWENKSKSGVGRCSMLIASNETWKKVECEHGFGRVVCKVPLGPDYTAIAIIVATLSILVLMGGLIWFLFQRHRLHLAGFSSVRYAQGVNEDEIMLPSFHD

SEQ ID NO: 16 - protein, 30 aa, Homo sapiens
EVQLVESGGGLVKPGGSLRLSCAASGFTYS

SEQ ID NO: 17 - protein, 14 aa, Homo sapiens
WVRQAPGKGLEWVG

SEQ ID NO: 18 - protein, 32 aa, Homo sapiens
RFTISRDDSKNTLYLQMNSLKTEDTAVYYCTI

SEQ ID NO: 19 - protein, 11 aa, Homo sapiens
WGQGTLVTVSS

SEQ ID NO: 20 - protein, 23 aa, Homo sapiens
DVQMTQSPSSLSASVGDRVTITC

SEQ ID NO: 21 - protein, 15 aa, Homo sapiens
WYQQRPGKAPNLLIY

SEQ ID NO: 22 - protein, 32 aa, Homo sapiens
GVPSRFSGSGSGTDFTLTISTLQPEDFATYYC

SEQ ID NO: 23 - protein, 11 aa, Homo sapiens
FGQGTKVEIKR

SEQ ID NO: 24 - protein, 10 aa, Homo sapiens
WEVKDCRSFK

SEQ ID NO: 25 - protein, 12 aa, Homo sapiens
PASLSCYKVFHA

SEQ ID NO: 26 - protein, 20 aa, Homo sapiens
PWRRGWHFYDDREFIYLRPF

SEQ ID NO: 27 - protein, 19 aa, Homo sapiens
DDHFTYSRYPWHRFPVTFG

SEQ ID NO: 28 - protein, 12 aa, Homo sapiens
RELTYSNFHPLL

SEQ ID NO: 29 - protein, 17 aa, Homo sapiens
FTSCSERHFVSLCQKYS

SEQ ID NO: 30 - protein, 12 aa, Homo sapiens
TVKYLNNLYKII

SEQ ID NO: 31 - protein, 11 aa, Homo sapiens
EAVYFHQHSIL

SEQ ID NO: 32 - protein, 11 aa, Homo sapiens
KKLSRLTYSSC

SEQ ID NO: 33 - protein, 20 aa, Homo sapiens
NGSRWIQYKGHCYKSDQALH

SEQ ID NO: 34 - protein, 25 aa, Homo sapiens
ISEWPIDDHFTYSRYPWHRFPVTFG

SEQ ID NO: 35 - protein, 20 aa, Homo sapiens
QTLQNASETVKYLNNLYKII

SEQ ID NO: 36 - protein, 10 aa, Homo sapiens
DDHFTYSRYP

SEQ ID NO: 37 - protein, 15 aa, Homo sapiens
FTSCSERHFVSLCQK

SEQ ID NO: 38 - protein, 451 aa, synthetic construct
  REGION 1..451: note = Rituximab VH sequence
QVQLQQPGAELVKPGASVKMSCKASGYTFTSYNMHWVKQTPGRGLEWIGAIYPGNGDTSYNQKFKGKATLTADKSSSTAYMQLSSLTSEDSAVYYCARSTYYGGDWYFNVWGAGTTVTVSAASTKGPSVFPLAPSSKSTSGGTAALGCLVKDYFPEPVTVSWNSGALTSGVHTFPAVLQSSGLYSLSSVVTVPSSSLGTQTYICNVNHKPSNTKVDKKAEPKSCDKTHTCPPCPAPELLGGPSVFLFPPKPKDTLMISRTPEVTCVVVDVSHEDPEVKFNWYVDGVEVHNAKTKPREEQYNSTYRVVSVLTVLHQDWLNGKEYKCKVSNKALPAPIEKTISKAKGQPREPQVYTLPPSRDELTKNQVSLTCLVKGFYPSDIAVEWESNGQPENNYKTTPPVLDSDGSFFLYSKLTVDKSRWQQGNVFSCSVMHEALHNHYTQKSLSLSPGK

SEQ ID NO: 39 - protein, 213 aa, synthetic construct
  REGION 1..213: note = Rituximab VL sequence
QIVLSQSPAILSASPGEKVTMTCRASSSVSYIHWFQQKPGSSPKPWIYATSNLASGVPVRFSGSGSGTSYSLTISRVEAEDAATYYCQQWTSNPPTFGGGTKLEIKRTVAAPSVFIFPPSDEQLKSGTASVVCLLNNFYPREAKVQWKVDNALQSGNSQESVTEQDSKDSTYSLSSTLTLSKADYEKHKVYACEVTHQGLSSPVTKSFNRGEC

SEQ ID NO: 40 - protein, 5 aa, synthetic construct
  REGION 1..5: note = Rituximab VH_CDR1
SYNMH

SEQ ID NO: 41 - protein, 17 aa, synthetic construct
  REGION 1..17: note = Rituximab VH_CDR2
AIYPGNGDTSYNQKFKG

SEQ ID NO: 42 - protein, 12 aa, synthetic construct
  REGION 1..12: note = Rituximab VH_CDR3
STYYGGDWYFNV

SEQ ID NO: 43 - protein, 10 aa, synthetic construct
  REGION 1..10: note = Rituximab VL_CDR1
RASSSVSYIH

SEQ ID NO: 44 - protein, 7 aa, synthetic construct
  REGION 1..7: note = Rituximab VL_CDR2
ATSNLAS

SEQ ID NO: 45 - protein, 10 aa, synthetic construct
  REGION 1..10: note = Rituximab VL_CDR3
QQWTSNPPTF

SEQ ID NO: 46 - protein, 8 aa, Homo sapiens
GWHFYDDR

SEQ ID NO: 47 - protein, 14 aa, Homo sapiens
ISEWPIDDHFTYSR

SEQ ID NO: 48 - protein, 15 aa, Homo sapiens
FPVTFGEECLYMSAK

SEQ ID NO: 49 - protein, 15 aa, Homo sapiens
ELTYSNFHPLLVSGR

SEQ ID NO: 50 - protein, 8 aa, Homo sapiens
HFVSLCQK

SEQ ID NO: 51 - protein, 11 aa, Homo sapiens
QTLQNASETVK

SEQ ID NO: 52 - protein, 4 aa, synthetic construct
  REGION 1..4: note = Linker
GFLG

SEQ ID NO: 53 - protein, 8 aa, synthetic construct
  REGION 1..8: note = Peptide
WEVKDCRS

SEQ ID NO: 54 - protein, 8 aa, synthetic construct
  REGION 1..8: note = Peptide
EVKDCRSF

SEQ ID NO: 55 - protein, 8 aa, synthetic construct
  REGION 1..8: note = Peptide
VKDCRSFK

SEQ ID NO: 56 - protein, 8 aa, synthetic construct
  REGION 1..8: note = Peptide
KDCRSFKA

SEQ ID NO: 57 - protein, 8 aa, synthetic construct
  REGION 1..8: note = Peptide
DCRSFKAL

SEQ ID NO: 58 - protein, 8 aa, synthetic construct
  REGION 1..8: note = Peptide
CRSFKALS

SEQ ID NO: 59 - protein, 8 aa, synthetic construct
  REGION 1..8: note = Peptide
RSFKALSI

SEQ ID NO: 60 - protein, 8 aa, synthetic construct
  REGION 1..8: note = Peptide
PASLSCYK

SEQ ID NO: 61 - protein, 8 aa, synthetic construct
  REGION 1..8: note = Peptide
ASLSCYKV

SEQ ID NO: 62 - protein, 8 aa, synthetic construct
  REGION 1..8: note = Peptide
SLSCYKVF

SEQ ID NO: 63 - protein, 8 aa, synthetic construct
  REGION 1..8: note = Peptide
LSCYKVFH

SEQ ID NO: 64 - protein, 8 aa, synthetic construct
  REGION 1..8: note = Peptide
SCYKVFHA

SEQ ID NO: 65 - protein, 8 aa, synthetic construct
  REGION 1..8: note = Peptide
CYKVFHAE

SEQ ID NO: 66 - protein, 8 aa, synthetic construct
  REGION 1..8: note = Peptide
YKVFHAER

SEQ ID NO: 67 - protein, 8 aa, synthetic construct
  REGION 1..8: note = Peptide
KVFHAERI

SEQ ID NO: 68 - protein, 8 aa, synthetic construct
  REGION 1..8: note = Peptide
VFHAERIV

SEQ ID NO: 69 - protein, 8 aa, synthetic construct
  REGION 1..8: note = Peptide
FHAERIVR

SEQ ID NO: 70 - protein, 8 aa, synthetic construct
  REGION 1..8: note = Peptide
DCAAVKVF

SEQ ID NO: 71 - protein, 8 aa, synthetic construct
  REGION 1..8: note = Peptide
AAVKVFHR

SEQ ID NO: 72 - protein, 8 aa, synthetic construct
  REGION 1..8: note = Peptide
VKVFHRPW

SEQ ID NO: 73 - protein, 8 aa, synthetic construct
  REGION 1..8: note = Peptide
VFHRPWRR

SEQ ID NO: 74 - protein, 8 aa, synthetic construct
  REGION 1..8: note = Peptide
HRPWRRGW

SEQ ID NO: 75 - protein, 8 aa, synthetic construct
  REGION 1..8: note = Peptide
PWRRGWHF

SEQ ID NO: 76 - protein, 8 aa, synthetic construct
  REGION 1..8: note = Peptide
RRGWHFYD

SEQ ID NO: 77 - protein, 8 aa, synthetic construct
  REGION 1..8: note = Peptide
GWHFYDDR

SEQ ID NO: 78 - protein, 8 aa, synthetic construct
  REGION 1..8: note = Peptide
HFYDDREF

SEQ ID NO: 79 - protein, 8 aa, synthetic construct
  REGION 1..8: note = Peptide
YDDREFIY

SEQ ID NO: 80 - protein, 8 aa, synthetic construct
  REGION 1..8: note = Peptide
DREFIYLR

SEQ ID NO: 81 - protein, 8 aa, synthetic construct
  REGION 1..8: note = Peptide
EFIYLRPF

SEQ ID NO: 82 - protein, 8 aa, synthetic construct
  REGION 1..8: note = Peptide
PIDDHFTY

SEQ ID NO: 83 - protein, 8 aa, synthetic construct
  REGION 1..8: note = Peptide
IDDHFTYS

SEQ ID NO: 84 - protein, 8 aa, synthetic construct
  REGION 1..8: note = Peptide
DDHFTYSR

SEQ ID NO: 85 - protein, 8 aa, synthetic construct
  REGION 1..8: note = Peptide
DHFTYSRY

SEQ ID NO: 86 - protein, 8 aa, synthetic construct
  REGION 1..8: note = Peptide
HFTYSRYP

SEQ ID NO: 87 - protein, 8 aa, synthetic construct
  REGION 1..8: note = Peptide
FTYSRYPW

SEQ ID NO: 88 - protein, 8 aa, synthetic construct
  REGION 1..8: note = Peptide
TYSRYPWH

SEQ ID NO: 89 - protein, 8 aa, synthetic construct
  REGION 1..8: note = Peptide
YSRYPWHR

SEQ ID NO: 90 - protein, 8 aa, synthetic construct
  REGION 1..8: note = Peptide
SRYPWHRF

SEQ ID NO: 91 - protein, 8 aa, synthetic construct
  REGION 1..8: note = Peptide
RYPWHRFP

SEQ ID NO: 92 - protein, 8 aa, synthetic construct
  REGION 1..8: note = Peptide
YPWHRFPV

SEQ ID NO: 93 - protein, 8 aa, synthetic construct
  REGION 1..8: note = Peptide
PWHRFPVT

SEQ ID NO: 94 - protein, 8 aa, synthetic construct
  REGION 1..8: note = Peptide
WHRFPVTF

SEQ ID NO: 95 - protein, 8 aa, synthetic construct
  REGION 1..8: note = Peptide
HRFPVTFG

SEQ ID NO: 96 - protein, 8 aa, synthetic construct
  REGION 1..8: note = Peptide
RELTYSNF

SEQ ID NO: 97 - protein, 8 aa, synthetic construct
  REGION 1..8: note = Peptide
ELTYSNFH

SEQ ID NO: 98 - protein, 8 aa, synthetic construct
  REGION 1..8: note = Peptide
LTYSNFHP

SEQ ID NO: 99 - protein, 8 aa, synthetic construct
  REGION 1..8: note = Peptide
TYSNFHPL

SEQ ID NO: 100 - protein, 8 aa, synthetic construct
  REGION 1..8: note = Peptide
YSNFHPLL

SEQ ID NO: 101 - protein, 8 aa, synthetic construct
  REGION 1..8: note = Peptide
SNFHPLLV

SEQ ID NO: 102 - protein, 8 aa, synthetic construct
  REGION 1..8: note = Peptide
NFHPLLVS

SEQ ID NO: 103 - protein, 8 aa, synthetic construct
  REGION 1..8: note = Peptide
FHPLLVSG

SEQ ID NO: 104 - protein, 8 aa, synthetic construct
  REGION 1..8: note = Peptide
HPLLVSGR

SEQ ID NO: 105 - protein, 8 aa, synthetic construct
  REGION 1..8: note = Peptide
PLLVSGRL

SEQ ID NO: 106 - protein, 8 aa, synthetic construct
  REGION 1..8: note = Peptide
LLVSGRLR

SEQ ID NO: 107 - protein, 8 aa, synthetic construct
  REGION 1..8: note = Peptide
LVSGRLRI

SEQ ID NO: 108 - protein, 8 aa, synthetic construct
  REGION 1..8: note = Peptide
VSGRLRIP

SEQ ID NO: 109 - protein, 8 aa, synthetic construct
  REGION 1..8: note = Peptide
FTSCSERH

SEQ ID NO: 110 - protein, 8 aa, synthetic construct
  REGION 1..8: note = Peptide
TSCSERHF

SEQ ID NO: 111 - protein, 8 aa, synthetic construct
  REGION 1..8: note = Peptide
SCSERHFV

SEQ ID NO: 112 - protein, 8 aa, synthetic construct
  REGION 1..8: note = Peptide
CSERHFVS

SEQ ID NO: 113 - protein, 8 aa, synthetic construct
  REGION 1..8: note = Peptide
SERHFVSL

SEQ ID NO: 114 - protein, 8 aa, synthetic construct
  REGION 1..8: note = Peptide
ERHFVSLC

SEQ ID NO: 115 - protein, 8 aa, synthetic construct
  REGION 1..8: note = Peptide
RHFVSLCQ

SEQ ID NO: 116 - protein, 8 aa, synthetic construct
  REGION 1..8: note = Peptide
HFVSLCQK

SEQ ID NO: 117 - protein, 8 aa, synthetic construct
  REGION 1..8: note = Peptide
FVSLCQKY

SEQ ID NO: 118 - protein, 8 aa, synthetic construct
  REGION 1..8: note = Peptide
VSLCQKYS

SEQ ID NO: 119 - protein, 8 aa, synthetic construct
  REGION 1..8: note = Peptide
SLCQKYSE

SEQ ID NO: 120 - protein, 8 aa, synthetic construct
  REGION 1..8: note = Peptide
LCQKYSEV

SEQ ID NO: 121 - protein, 8 aa, synthetic construct
  REGION 1..8: note = Peptide
CQKYSEVK

SEQ ID NO: 122 - protein, 8 aa, synthetic construct
  REGION 1..8: note = Peptide
QKYSEVKS

SEQ ID NO: 123 - protein, 8 aa, synthetic construct
  REGION 1..8: note = Peptide
TVKYLNNL

SEQ ID NO: 124 - protein, 8 aa, synthetic construct
  REGION 1..8: note = Peptide
VKYLNNLY

SEQ ID NO: 125 - protein, 8 aa, synthetic construct
  REGION 1..8: note = Peptide
KYLNNLYK

SEQ ID NO: 126 - protein, 8 aa, synthetic construct
  REGION 1..8: note = Peptide
YLNNLYKI

SEQ ID NO: 127 - protein, 8 aa, synthetic construct
  REGION 1..8: note = Peptide
LNNLYKII

SEQ ID NO: 128 - protein, 8 aa, synthetic construct
  REGION 1..8: note = Peptide
NNLYKIIP

SEQ ID NO: 129 - protein, 8 aa, synthetic construct
  REGION 1..8: note = Peptide
NLYKIIPK

SEQ ID NO: 130 - protein, 8 aa, synthetic construct
  REGION 1..8: note = Peptide
LYKIIPKT

SEQ ID NO: 131 - protein, 8 aa, synthetic construct
  REGION 1..8: note = Peptide
YKIIPKTL

SEQ ID NO: 132 - protein, 8 aa, synthetic construct
  REGION 1..8: note = Peptide
KIIPKTLT

SEQ ID NO: 133 - protein, 8 aa, synthetic construct
  REGION 1..8: note = Peptide
IIPKTLTW

SEQ ID NO: 134 - protein, 8 aa, synthetic construct
  REGION 1..8: note = Peptide
IPKTLTWH

SEQ ID NO: 135 - protein, 8 aa, synthetic construct
  REGION 1..8: note = Peptide
PKTLTWHS

SEQ ID NO: 136 - protein, 8 aa, synthetic construct
  REGION 1..8: note = Peptide
KTLTWHSA

SEQ ID NO: 137 - protein, 8 aa, synthetic construct
  REGION 1..8: note = Peptide
TLTWHSAK

SEQ ID NO: 138 - protein, 8 aa, synthetic construct
  REGION 1..8: note = Peptide
EAVYFHQH

SEQ ID NO: 139 - protein, 8 aa, synthetic construct
  REGION 1..8: note = Peptide
AVYFHQHS

SEQ ID NO: 140 - protein, 8 aa, synthetic construct
  REGION 1..8: note = Peptide
VYFHQHSI

SEQ ID NO: 141 - protein, 8 aa, synthetic construct
  REGION 1..8: note = Peptide
YFHQHSIL

SEQ ID NO: 142 - protein, 8 aa, synthetic construct
  REGION 1..8: note = Peptide
FHQHSILA

SEQ ID NO: 143 - protein, 8 aa, synthetic construct
  REGION 1..8: note = Peptide
KKLSRLTY

SEQ ID NO: 144 - protein, 8 aa, synthetic construct
  REGION 1..8: note = Peptide
KLSRLTYS

SEQ ID NO: 145 - protein, 8 aa, synthetic construct
  REGION 1..8: note = Peptide
LSRLTYSS

SEQ ID NO: 146 - protein, 8 aa, synthetic construct
  REGION 1..8: note = Peptide
SRLTYSSR

SEQ ID NO: 147 - protein, 8 aa, synthetic construct
  REGION 1..8: note = Peptide
RLTYSSRC

SEQ ID NO: 148 - protein, 8 aa, synthetic construct
  REGION 1..8: note = Peptide
NGSRWIQY

SEQ ID NO: 149 - protein, 8 aa, synthetic construct
  REGION 1..8: note = Peptide
GSRWIQYK

SEQ ID NO: 150 - protein, 8 aa, synthetic construct
  REGION 1..8: note = Peptide
SRWIQYKG

SEQ ID NO: 151 - protein, 8 aa, synthetic construct
  REGION 1..8: note = Peptide
RWIQYKGH

SEQ ID NO: 152 - protein, 8 aa, synthetic construct
  REGION 1..8: note = Peptide
WIQYKGHC

SEQ ID NO: 153 - protein, 8 aa, synthetic construct
  REGION 1..8: note = Peptide
IQYKGHCY

SEQ ID NO: 154 - protein, 8 aa, synthetic construct
  REGION 1..8: note = Peptide
QYKGHCYK

SEQ ID NO: 155 - protein, 8 aa, synthetic construct
  REGION 1..8: note = Peptide
YKGHCYKS

SEQ ID NO: 156 - protein, 8 aa, synthetic construct
  REGION 1..8: note = Peptide
KGHCYKSD

SEQ ID NO: 157 - protein, 8 aa, synthetic construct
  REGION 1..8: note = Peptide
GHCYKSDQ

SEQ ID NO: 158 - protein, 8 aa, synthetic construct
  REGION 1..8: note = Peptide
HCYKSDQA

SEQ ID NO: 159 - protein, 8 aa, synthetic construct
  REGION 1..8: note = Peptide
CYKSDQAL

SEQ ID NO: 160 - protein, 8 aa, synthetic construct
  REGION 1..8: note = Peptide
YKSDQALH

SEQ ID NO: 161 - protein, 8 aa, synthetic construct
  REGION 1..8: note = Peptide
KSDQALHS

SEQ ID NO: 162 - protein, 8 aa, synthetic construct
  REGION 1..8: note = Peptide
SDQALHSF

SEQ ID NO: 163 - protein, 8 aa, synthetic construct
  REGION 1..8: note = Peptide
DQALHSFS

SEQ ID NO: 164 - protein, 1722 aa, Homo sapiens; identical to SEQ ID NO: 15

SEQ ID NO: 165 - protein, 23 aa, synthetic construct
  REGION 1..23: note = Peptide
CIKPVYGWIVADDCDETEDKLWK

SEQ ID NO: 166 - protein, 11 aa, synthetic construct
  REGION 1..11: note = Peptide
CEHHSLYGAAR

SEQ ID NO: 167 - protein, 34 aa, synthetic construct
  REGION 1..34: note = Peptide
DGHGTAISNASDVWKKGGSEESLCDQPYHEIYTR

SEQ ID NO: 168 - protein, 19 aa, synthetic construct
  REGION 1..19: note = Peptide
KGGSEESLCDQPYHEIYTR

SEQ ID NO: 169 - protein, 18 aa, synthetic construct
  REGION 1..18: note = Peptide
GGSEESLCDQPYHEIYTR

SEQ ID NO: 170 - protein, 15 aa, synthetic construct
  REGION 1..15: note = Peptide
DGHGTAISNASDVWK

SEQ ID NO: 171 - protein, 17 aa, synthetic construct
  REGION 1..17: note = Peptide
WGICLKPENGCEDNWEK

SEQ ID NO: 172 - protein, 13 aa, synthetic construct
  REGION 1..13: note = Peptide
IFWIGLNQLYSAR

SEQ ID NO: 173 - protein, 15 aa, synthetic construct
  REGION 1..15: note = Peptide
LHNEDIKEEVWIGLK

SEQ ID NO: 174 - protein, 15 aa, synthetic construct
  REGION 1..15: note = Peptide
TPNCVSYLGELGQWK

SEQ ID NO: 175 - protein, 23 aa, synthetic construct
  REGION 1..23: note = Peptide
YFWTGLRDVDSCGEYNWATVGGR

SEQ ID NO: 176 - protein, 11 aa, synthetic construct
  REGION 1..11: note = Peptide
SVGKWEVKDCR

SEQ ID NO: 177 - protein, 10 aa, synthetic construct
  REGION 1..10: note = Peptide
WEVKDCRSFK

SEQ ID NO: 178 - protein, 7 aa, synthetic construct
  REGION 1..7: note = Peptide
ALSICKK

SEQ ID NO: 179 - protein, 12 aa, synthetic construct
  REGION 1..12: note = Peptide
PASLSCYKVFHA

SEQ ID NO: 180 - protein, 8 aa, synthetic construct
  REGION 1..8: note = Peptide
RNWEEAER

SEQ ID NO: 181 - protein, 33 aa, synthetic construct
  REGION 1..33: note = Peptide
RSPDLQGSWQWSDRTPVSTIIMPNEFQQDYDIR

SEQ ID NO: 182 - protein, 19 aa, synthetic construct
  REGION 1..19: note = Peptide
TPVSTIIMPNEFQQDYDIR

SEQ ID NO: 183 - protein, 20 aa, synthetic construct
  REGION 1..20: note = Peptide
PWRRGWHFYDDREFIYLRPF

SEQ ID NO: 184 - protein, 8 aa, synthetic construct
  REGION 1..8: note = Peptide
GWHFYDDR

SEQ ID NO: 185 - protein, 14 aa, synthetic construct
  REGION 1..14: note = Peptide
ISEWPIDDHFTYSR

SEQ ID NO: 186 - protein, 19 aa, synthetic construct
  REGION 1..19: note = Peptide
DDHFTYSRYPWHRFPVTFG

SEQ ID NO: 187 - protein, 30 aa, synthetic construct
  REGION 1..30: note = Peptide
FPVTFGEECLYMSAKTWLIDLGKPTDCSTK

SEQ ID NO: 188 - protein, 15 aa, synthetic construct
  REGION 1..15: note = Peptide
TWLIDLGKPTDCSTK

SEQ ID NO: 189 - protein, 8 aa, synthetic construct
  REGION 1..8: note = Peptide
YNVSSLEK

SEQ ID NO: 190 - protein, 12 aa, synthetic construct
  REGION 1..12: note = Peptide
VQCSEQWIPFQN

SEQ ID NO: 191 - protein, 12 aa, synthetic construct
  REGION 1..12: note = Peptide
RELTYSNFHPLL

SEQ ID NO: 192 - protein, 39 aa, synthetic construct
  REGION 1..39: note = Peptide
ELTYSNFHPLLVSGRLRIPENFFEEESRYHCALILNLQK

SEQ ID NO: 193 - protein, 11 aa, synthetic construct
  REGION 1..11: note = Peptide
YHCALILNLQK

SEQ ID NO: 194 - protein, 17 aa, synthetic construct
  REGION 1..17: note = Peptide
FTSCSERHFVSLCQKYS

SEQ ID NO: 195 - protein, 8 aa, synthetic construct
  REGION 1..8: note = Peptide
HFVSLCQK

SEQ ID NO: 196 - protein, 11 aa, synthetic construct
  REGION 1..11: note = Peptide
QTLQNASETVK

SEQ ID NO: 197 - protein, 12 aa, synthetic construct
  REGION 1..12: note = Peptide
TVKYLNNLYKII

SEQ ID NO: 198 - protein, 8 aa, synthetic construct
  REGION 1..8: note = Peptide
TLTWHSAK

SEQ ID NO: 199 - protein, 14 aa, synthetic construct
  REGION 1..14: note = Peptide
NRHMATTQDEVHTK

SEQ ID NO: 200 - protein, 7 aa, synthetic construct
  REGION 1..7: note = Peptide
SHILSIR

SEQ ID NO: 201 - protein, 16 aa, synthetic construct
  REGION 1..16: note = Peptide
SLMWFDKTPLSYTHWR

SEQ ID NO: 202 - protein, 7 aa, synthetic construct
  REGION 1..7: note = Peptide
SLMWFDK

SEQ ID NO: 203 - protein, 11 aa, synthetic construct
  REGION 1..11: note = Peptide
EAVYFHQHSIL

SEQ ID NO: 204 - protein, 10 aa, synthetic construct
  REGION 1..10: note = Peptide
KKLSRLTYSS

SEQ ID NO: 205 - protein, 20 aa, synthetic construct
  REGION 1..20: note = Peptide
NGSRWIQYKGHCYKSDQALH

SEQ ID NO: 206 - protein, 21 aa, synthetic construct
  REGION 1..21: note = Peptide
HDHSATIVSIKDEDENKFVSR

SEQ ID NO: 207 - protein, 9 aa, synthetic construct
  REGION 1..9: note = Peptide
VECEHGFGR